European Patent Specification EP 3 568 147 B1, published May 1, 2024. Title: PEPTIDE. Applicant: Rogers, April. Application PCT/. The sequence listing filed with the application follows.

SEQUENCE LISTING (7 sequences)

SEQ ID NO: 1 - protein, 15 aa, Artificial
  Peptide
VPSVPIQQFPTEDWS

SEQ ID NO: 2 - protein, 16 aa, Artificial
  Peptide
CVPSVPIQQFPTEDWS

SEQ ID NO: 3 - protein, 32 aa, Artificial
  Peptide
CVPSVPIQQFPTEDWSCVPSVPIQQFPTEDWS

SEQ ID NO: 4 - DNA, 45 bp, Artificial
  Peptide
gtgcccagcgtgcccatccagcagttccccaccgaggactggagc

SEQ ID NO: 5 - DNA, 48 bp, Artificial
  Peptide
tgcgtgcccagcgtgcccatccagcagttccccaccgaggactggagc

SEQ ID NO: 6 - protein, 295 aa, Homo sapiens [sequence omitted]

SEQ ID NO: 7 - DNA, 885 bp, Homo sapiens
atgagcggcgccctggacgtgctgcagatgaaggaggaggacgtgctgaagttcctggccgccggcacccacctgggcggcaccaacctggacttccagatggagcagtacatctacaagaggaagagcgacggcatctacatcatcaacctgaagaggacctgggagaagctgctgctggccgccagggccatcgtggccatcgagaaccccgccgacgtgagcgtgatcagcagcaggaacaccggccagagggccgtgctgaagttcgccgccgccaccggcgccacccccatcgccggcaggttcacccccggcaccttcaccaaccagatccaggccgccttcagggagcccaggctgctggtggtgaccgaccccagggccgaccaccagcccctgaccgaggccagctacgtgaacctgcccaccatcgccctgtgcaacaccgacagccccctgaggtacgtggacatcgccatcccctgcaacaacaagggcgcccacagcgtgggcctgatgtggtggatgctggccagggaggtgctgaggatgaggggcaccatcagcagggagcacccctgggaggtgatgcccgacctgtacttctacagggaccccgaggagatcgagaaggaggagcaggccgccgccgagaaggccgtgaccaaggaggagttccagggcgagtggaccgcccccgcccccgagttcaccgccacccagcccgaggtggccgactggagcgagggcgtgcaggtgcccagcgtgcccatccagcagttccccaccgaggactggagcgcccagcccgccaccgaggactggagcgccgcccccaccgcccaggccaccgagtgggtgggcgccaccaccgactggagc